European Patent Application EP 4 134 451 A1, published February 15, 2023. Title: METHOD FOR IDENTIFYING RESPONSIVENESS TO FIBROBLAST GROWTH FACTOR RECEPTOR 1 INHIBITOR THERAPY. Applicant: Universität zu Köln. The sequence listing filed with the application follows.

SEQUENCE LISTING (37 sequences)

SEQ ID NO: 1 - protein, 822 aa, Homo sapiens [sequence omitted]

SEQ ID NO: 2 - DNA, 2936 bp, Homo sapiens
gtgggagagtgacacacaaaacaccccgggaagccggaggaggcgtggaaaggtggggcccgggaggtaaaactgggatcggcgcgttcagtgaggctgattaaagaacaacgcgcaaccagcgccatacggcgctcctcagggtgactcggctctctagctcttaagggttagaagcgaccctcgcacggtccccggtgccacctggagcatcataatggactctgtggtgccctctgacaagggcaactacacctgcattgtggagaatgagtacggcagcatcaaccacacataccagctggatgtcgtggagcggtcccctcaccggcccatcctgcaagcagggttgcccgccaacaaaacagtggccctgggtagcaacgtggagttcatgtgtaaggtgtacagtgacccgcagccgcacatccagtggctaaagcacatcgaggtgaatgggagcaagattggcccagacaacctgccttatgtccagatcttgaagactgctggagttaataccaccgacaaagagatggaggtgcttcacttaagaaatgtctcctttgaggacgcaggggagtatacgtgcttggcgggtaactctatcggactctcccatcactctgcatggttgaccgttctggaagccctggaagagaggccggcagtgatgacctcgcccctgtacctggagatcatcatctattgcacaggggccttcctcatctcctgcatggtggggtcggtcatcgtctacaagatgaagagtggtaccaagaagagtgacttccacagccagatggctgtgcacaagctggccaagagcatccctctgcgcagacaggtaacagtgtctgctgactccagtgcatccatgaactctggggttcttctggttcggccatcacggctctcctccagtgggactcccatgctagcaggggtctctgagtatgagcttcccgaagaccctcgctgggagctgcctcgggacagactggtcttaggcaaacccctgggagagggctgctttgggcaggtggtgttggcagaggctatcgggctggacaaggacaaacccaaccgtgtgaccaaagtggctgtgaagatgttgaagtcggacgcaacagagaaagacttgtcagacctgatctcagaaatggagatgatgaagatgatcgggaagcataagaatatcatcaacctgctgggggcctgcacgcaggatggtcccttgtatgtcatcgtggagtatgcctccaagggcaacctgcgggagtacctgcaggcccggaggcccccagggctggaatactgctacaaccccagccacaacccagaggagcagctctcctccaaggacctggtgtcctgcgcctaccaggtggcccgaggcatggagtatctggcctccaagaagtgcatacaccgagacctggcagccaggaatgtcctggtgacagaggacaatgtgatgaagatagcagactttggcctcgcacgggacattcaccacatcgactactataaaaagacaaccaacggccgactgcctgtgaagtggatggcacccgaggcattatttgaccggatctacacccaccagagtgatgtgtggtctttcggggtgctcctgtgggagatcttcactctgggcggctccccataccccggtgtgcctgtggaggaacttttcaagctgctgaaggagggtcaccgcatggacaagcccagtaactgcaccaacgagctgtacatgatgatgcgggactgctggcatgcagtgccctcacagagacccaccttcaagcagctggtggaagacctggaccgcatcgtggccttgacctccaaccaggagtacctggacctgtccatgcccctggaccagtactcccccagctttcccgacacccggagctctacgtgctcctcaggggaggattccgtcttctctcatgagccgctgcccgaggagccctgcctgccccgacacccagcccagcttgccaatggcggactcaaacgccgctgactgccacccacacgccctccccagactccaccgtcagctgtaaccctcacccacagcccctgctgggcccaccacctgtccgtccctgtcccctttcctgctggcaggagccggctgcctaccaggggccttcctgtgtggcctgccttcaccccactcagctcacctctccctccacctcctctccacctgctggtgagaggtgcaaagaggcagatctttgctgccagccacttcatcccctcccagatgttggaccaacacccctccctgccaccaggcactgcctggagggcagggagtgggagccaatgaacaggcatgcaagtgagagcttcctgagctttctcctgtcggtttggtctgttttgccttcacccataagcccctcgcactctggtggcaggtgccttgtcctcagggctacagcagtagggaggtcagtgcttcgtgcctcgattgaaggtgacctctgccccagataggtggtgccagtggcttattaattccgatactagtttgctttgctgaccaaatgcctggtaccagaggatggtgaggcgaaggccaggttgggggcagtgttgtggccctggggcccagccccaaactgggggctctgtatatagctatgaagaaaacacaaagtgtataaatctgagtatatatttacatgtctttttaaaagggtcgttaccagagatttacccatcgggtaagatgctcctggtggctgggaggcatcagttgctatatattaaaaacaaaaaagaaaaaaaaggaaaatgtttttaaaaaggtcatatattttttgctacttttgctgttttatttttttaaattatgttctaaacctattttcagtttaggtccctcaataaaaattgctgctgcttca

SEQ ID NO: 3 - DNA, 1821 bp, Homo sapiens
atggactctgtggtgccctctgacaagggcaactacacctgcattgtggagaatgagtacggcagcatcaaccacacataccagctggatgtcgtggagcggtcccctcaccggcccatcctgcaagcagggttgcccgccaacaaaacagtggccctgggtagcaacgtggagttcatgtgtaaggtgtacagtgacccgcagccgcacatccagtggctaaagcacatcgaggtgaatgggagcaagattggcccagacaacctgccttatgtccagatcttgaagactgctggagttaataccaccgacaaagagatggaggtgcttcacttaagaaatgtctcctttgaggacgcaggggagtatacgtgcttggcgggtaactctatcggactctcccatcactctgcatggttgaccgttctggaagccctggaagagaggccggcagtgatgacctcgcccctgtacctggagatcatcatctattgcacaggggccttcctcatctcctgcatggtggggtcggtcatcgtctacaagatgaagagtggtaccaagaagagtgacttccacagccagatggctgtgcacaagctggccaagagcatccctctgcgcagacaggtaacagtgtctgctgactccagtgcatccatgaactctggggttcttctggttcggccatcacggctctcctccagtgggactcccatgctagcaggggtctctgagtatgagcttcccgaagaccctcgctgggagctgcctcgggacagactggtcttaggcaaacccctgggagagggctgctttgggcaggtggtgttggcagaggctatcgggctggacaaggacaaacccaaccgtgtgaccaaagtggctgtgaagatgttgaagtcggacgcaacagagaaagacttgtcagacctgatctcagaaatggagatgatgaagatgatcgggaagcataagaatatcatcaacctgctgggggcctgcacgcaggatggtcccttgtatgtcatcgtggagtatgcctccaagggcaacctgcgggagtacctgcaggcccggaggcccccagggctggaatactgctacaaccccagccacaacccagaggagcagctctcctccaaggacctggtgtcctgcgcctaccaggtggcccgaggcatggagtatctggcctccaagaagtgcatacaccgagacctggcagccaggaatgtcctggtgacagaggacaatgtgatgaagatagcagactttggcctcgcacgggacattcaccacatcgactactataaaaagacaaccaacggccgactgcctgtgaagtggatggcacccgaggcattatttgaccggatctacacccaccagagtgatgtgtggtctttcggggtgctcctgtgggagatcttcactctgggcggctccccataccccggtgtgcctgtggaggaacttttcaagctgctgaaggagggtcaccgcatggacaagcccagtaactgcaccaacgagctgtacatgatgatgcgggactgctggcatgcagtgccctcacagagacccaccttcaagcagctggtggaagacctggaccgcatcgtggccttgacctccaaccaggagtacctggacctgtccatgcccctggaccagtactcccccagctttcccgacacccggagctctacgtgctcctcaggggaggattccgtcttctctcatgagccgctgcccgaggagccctgcctgccccgacacccagcccagcttgccaatggcggactcaaacgccgctga

SEQ ID NO: 4 - DNA, 21 bp, Homo sapiens
cacctggagcatcataatgga

SEQ ID NO: 5 - DNA, 22 bp, Homo sapiens
tggagcatcataatggactctg

SEQ ID NO: 6 - DNA, 19 bp, Homo sapiens
agtcagcggcgtttgagtc

SEQ ID NO: 7 - DNA, 18 bp, Homo sapiens
gtgtgggtggcagtcagc

SEQ ID NO: 8 - DNA, 19 bp, Homo sapiens
cagtcagcggcgtttgagt

SEQ ID NO: 9 - protein, 604 aa, Homo sapiens [sequence omitted]

SEQ ID NO: 10 - DNA, 2280 bp, Homo sapiens
ccctggaagagaggccggcagtgatgacctcgcccctgtacctggagatcatcatctattgcacaggggccttcctcatctcctgcatggtggggtcggtcatcgtctacaagatgaagagtggtaccaagaagagtgacttccacagccagatggctgtgcacaagctggccaagagcatccctctgcgcagacaggtgtctgctgactccagtgcatccatgaactctggggttcttctggttcggccatcacggctctcctccagtgggactcccatgctagcaggggtctctgagtatgagcttcccgaagaccctcgctgggagctgcctcgggacagactggtcttaggcaaacccctgggagagggctgctttgggcaggtggtgttggcagaggctatcgggctggacaaggacaaacccaaccgtgtgaccaaagtggctgtgaagatgttgaagtcggacgcaacagagaaagacttgtcagacctgatctcagaaatggagatgatgaagatgatcgggaagcataagaatatcatcaacctgctgggggcctgcacgcaggatggtcccttgtatgtcatcgtggagtatgcctccaagggcaacctgcgggagtacctgcaggcccggaggcccccagggctggaatactgctacaaccccagccacaacccagaggagcagctctcctccaaggacctggtgtcctgcgcctaccaggtggcccgaggcatggagtatctggcctccaagaagtgcatacaccgagacctggcagccaggaatgtcctggtgacagaggacaatgtgatgaagatagcagactttggcctcgcacgggacattcaccacatcgactactataaaaagacaaccaacggccgactgcctgtgaagtggatggcacccgaggcattatttgaccggatctacacccaccagagtgatgtgtggtctttcggggtgctcctgtgggagatcttcactctgggcggctccccataccccggtgtgcctgtggaggaacttttcaagctgctgaaggagggtcaccgcatggacaagcccagtaactgcaccaacgagctgtacatgatgatgcgggactgctggcatgcagtgccctcacagagacccaccttcaagcagctggtggaagacctggaccgcatcgtggccttgacctccaaccaggagtacctggacctgtccatgcccctggaccagtactcccccagctttcccgacacccggagctctacgtgctcctcaggggaggattccgtcttctctcatgagccgctgcccgaggagccctgcctgccccgacacccagcccagcttgccaatggcggactcaaacgccgctgactgccacccacacgccctccccagactccaccgtcagctgtaaccctcacccacagcccctgctgggcccaccacctgtccgtccctgtcccctttcctgctggcaggagccggctgcctaccaggggccttcctgtgtggcctgccttcaccccactcagctcacctctccctccacctcctctccacctgctggtgagaggtgcaaagaggcagatctttgctgccagccacttcatcccctcccagatgttggaccaacacccctccctgccaccaggcactgcctggagggcagggagtgggagccaatgaacaggcatgcaagtgagagcttcctgagctttctcctgtcggtttggtctgttttgccttcacccataagcccctcgcactctggtggcaggtgccttgtcctcagggctacagcagtagggaggtcagtgcttcgtgcctcgattgaaggtgacctctgccccagataggtggtgccagtggcttattaattccgatactagtttgctttgctgaccaaatgcctggtaccagaggatggtgaggcgaaggccaggttgggggcagtgttgtggccctggggcccagccccaaactgggggctctgtatatagctatgaagaaaacacaaagtgtataaatctgagtatatatttacatgtctttttaaaagggtcgttaccagagatttacccatcgggtaagatgctcctggtggctgggaggcatcagttgctatatattaaaaacaaaaaagaaaaaaaaggaaaatgtttttaaaaaggtcatatattttttgctacttttgctgttttatttttttaaattatgttctaaacctattttcagtttaggtccctcaataaaaattgctgctgcttca

SEQ ID NO: 11 - DNA, 1359 bp, Homo sapiens
atgacctcgcccctgtacctggagatcatcatctattgcacaggggccttcctcatctcctgcatggtggggtcggtcatcgtctacaagatgaagagtggtaccaagaagagtgacttccacagccagatggctgtgcacaagctggccaagagcatccctctgcgcagacaggtgtctgctgactccagtgcatccatgaactctggggttcttctggttcggccatcacggctctcctccagtgggactcccatgctagcaggggtctctgagtatgagcttcccgaagaccctcgctgggagctgcctcgggacagactggtcttaggcaaacccctgggagagggctgctttgggcaggtggtgttggcagaggctatcgggctggacaaggacaaacccaaccgtgtgaccaaagtggctgtgaagatgttgaagtcggacgcaacagagaaagacttgtcagacctgatctcagaaatggagatgatgaagatgatcgggaagcataagaatatcatcaacctgctgggggcctgcacgcaggatggtcccttgtatgtcatcgtggagtatgcctccaagggcaacctgcgggagtacctgcaggcccggaggcccccagggctggaatactgctacaaccccagccacaacccagaggagcagctctcctccaaggacctggtgtcctgcgcctaccaggtggcccgaggcatggagtatctggcctccaagaagtgcatacaccgagacctggcagccaggaatgtcctggtgacagaggacaatgtgatgaagatagcagactttggcctcgcacgggacattcaccacatcgactactataaaaagacaaccaacggccgactgcctgtgaagtggatggcacccgaggcattatttgaccggatctacacccaccagagtgatgtgtggtctttcggggtgctcctgtgggagatcttcactctgggcggctccccataccccggtgtgcctgtggaggaacttttcaagctgctgaaggagggtcaccgcatggacaagcccagtaactgcaccaacgagctgtacatgatgatgcgggactgctggcatgcagtgccctcacagagacccaccttcaagcagctggtggaagacctggaccgcatcgtggccttgacctccaaccaggagtacctggacctgtccatgcccctggaccagtactcccccagctttcccgacacccggagctctacgtgctcctcaggggaggattccgtcttctctcatgagccgctgcccgaggagccctgcctgccccgacacccagcccagcttgccaatggcggactcaaacgccgctga

SEQ ID NO: 12 - DNA, 18 bp, Homo sapiens
ccggcagtgatgacctcg

SEQ ID NO: 13 - DNA, 18 bp, Homo sapiens
cagtgatgacctcgcccc

SEQ ID NO: 14 - protein, 462 aa, Homo sapiens
MTSPLYLEIIIYCTGAFLISCMVGSVIVYKMKSGTKKSDFHSQMAVHKLAKSIPLRRQVSADSSASMNSGVLLVRPSRLSSSGTPMLAGVSEYELPEDPRWELPRDRLVLGKPLGEGCFGQVVLAEAIGLDKDKPNRVTKVAVKMLKSDATEKDLSDLISEMEMMKMIGKHKNIINLLGACTQDGPLYVIVEYASKGNLREYLQARRPPGLEYCYNPSHNPEEQLSSKDLVSCAYQVARGMEYLASKKCIHRDLAARNVLVTEDNVMKIADFGLARDIHHIDYYKKTTNGRLPVKWMAPEALFDRIYTHQSDVWSFGVLLWEIFTLGGSPYPGVPVEELFKLLKEGHRMDKPSNCTNELYMMMRDCWHAVPSQRPTFKQLVEDLDRIVALTSNQVLHPDLTTHLLPLRCFWKVRKRRCLLRGQEPHPCSRGAGQRVKAQQPSTMDGFLQGNRWGWAGEGAPT

SEQ ID NO: 15 - DNA, 2913 bp, Homo sapiens
ccgtagctccatattggacatccccagaaaagatggaaaagaaattgcatgcagtgccggctgccaagacagtgaagttcaaatgcccttccagtgggaccccaaaccccacactgcgctggttgaaaaatggcaaagaattcaaacctgaccacagaattggaggctacaaggtccgttatgccacctggagcatcataatggactctgtggtgccctctgacaagggcaactacacctgcattgtggagaatgagtacggcagcatcaaccacacataccagctggatgtcgtggagcggtcccctcaccggcccatcctgcaagcagggttgcccgccaacaaaacagtggccctgggtagcaacgtggagttcatgtgtaaggtgtacagtgacccgcagccgcacatccagtggctaaagcacatcgaggtgaatgggagcaagattggcccagacaacctgccttatgtccagatcttgaagactgctggagttaataccaccgacaaagagatggaggtgcttcacttaagaaatgtctcctttgaggacgcaggggagtatacgtgcttggcgggtaactctatcggactctcccatcactctgcatggttgaccgttctggaagccctggaagagaggccggcagtgatgacctcgcccctgtacctggagatcatcatctattgcacaggggccttcctcatctcctgcatggtggggtcggtcatcgtctacaagatgaagagtggtaccaagaagagtgacttccacagccagatggctgtgcacaagctggccaagagcatccctctgcgcagacaggtgtctgctgactccagtgcatccatgaactctggggttcttctggttcggccatcacggctctcctccagtgggactcccatgctagcaggggtctctgagtatgagcttcccgaagaccctcgctgggagctgcctcgggacagactggtcttaggcaaacccctgggagagggctgctttgggcaggtggtgttggcagaggctatcgggctggacaaggacaaacccaaccgtgtgaccaaagtggctgtgaagatgttgaagtcggacgcaacagagaaagacttgtcagacctgatctcagaaatggagatgatgaagatgatcgggaagcataagaatatcatcaacctgctgggggcctgcacgcaggatggtcccttgtatgtcatcgtggagtatgcctccaagggcaacctgcgggagtacctgcaggcccggaggcccccagggctggaatactgctacaaccccagccacaacccagaggagcagctctcctccaaggacctggtgtcctgcgcctaccaggtggcccgaggcatggagtatctggcctccaagaagtgcatacaccgagacctggcagccaggaatgtcctggtgacagaggacaatgtgatgaagatagcagactttggcctcgcacgggacattcaccacatcgactactataaaaagacaaccaacggccgactgcctgtgaagtggatggcacccgaggcattatttgaccggatctacacccaccagagtgatgtgtggtctttcggggtgctcctgtgggagatcttcactctgggcggctccccataccccggtgtgcctgtggaggaacttttcaagctgctgaaggagggtcaccgcatggacaagcccagtaactgcaccaacgagctgtacatgatgatgcgggactgctggcatgcagtgccctcacagagacccaccttcaagcagctggtggaagacctggaccgcatcgtggccttgacctccaaccaggagtacctggacctgtccatgcccctggaccagtactcccccagctttcccgacacccggagctctacgtgctcctcaggggaggattccgtcttctctcatgagccgctgcccgaggagccctgcctgccccgacacccagcccagcttgccaatggcggactcaaacgccgctgactgccacccacacgccctccccagactccaccgtcagctgtaaccctcacccacagcccctgctgggcccaccacctgtccgtccctgtcccctttcctgctggcaggagccggctgcctaccaggggccttcctgtgtggcctgccttcaccccactcagctcacctctccctccacctcctctccacctgctggtgagaggtgcaaagaggcagatctttgctgccagccacttcatcccctcccagatgttggaccaacacccctccctgccaccaggcactgcctggagggcagggagtgggagccaatgaacaggcatgcaagtgagagcttcctgagctttctcctgtcggtttggtctgttttgccttcacccataagcccctcgcactctggtggcaggtgccttgtcctcagggctacagcagtagggaggtcagtgcttcgtgcctcgattgaaggtgacctctgccccagataggtggtgccagtggcttattaattccgatactagtttgctttgctgaccaaatgcctggtaccagaggatggtgaggcgaaggccaggttgggggcagtgttgtggccctggggcccagccccaaactgggggctctgtatatagctatgaagaaaacacaaagtgtataaatctgagtatatatttacatgtctttttaaaagggtcgttaccagagatttacccatcgggtaagatgctcctggtggctgggaggcatcagttgctatatattaaaaacaaaaaagaaaaaaaaggaaaatgtttttaaaaaggtcatatattttttgctacttttgctgttttatttttttaaattatgttctaaacctattttcagtttaggtccctcaataaaaattgctgctgcttca

SEQ ID NO: 16 - DNA, 1983 bp, Homo sapiens
atggaaaagaaattgcatgcagtgccggctgccaagacagtgaagttcaaatgcccttccagtgggaccccaaaccccacactgcgctggttgaaaaatggcaaagaattcaaacctgaccacagaattggaggctacaaggtccgttatgccacctggagcatcataatggactctgtggtgccctctgacaagggcaactacacctgcattgtggagaatgagtacggcagcatcaaccacacataccagctggatgtcgtggagcggtcccctcaccggcccatcctgcaagcagggttgcccgccaacaaaacagtggccctgggtagcaacgtggagttcatgtgtaaggtgtacagtgacccgcagccgcacatccagtggctaaagcacatcgaggtgaatgggagcaagattggcccagacaacctgccttatgtccagatcttgaagactgctggagttaataccaccgacaaagagatggaggtgcttcacttaagaaatgtctcctttgaggacgcaggggagtatacgtgcttggcgggtaactctatcggactctcccatcactctgcatggttgaccgttctggaagccctggaagagaggccggcagtgatgacctcgcccctgtacctggagatcatcatctattgcacaggggccttcctcatctcctgcatggtggggtcggtcatcgtctacaagatgaagagtggtaccaagaagagtgacttccacagccagatggctgtgcacaagctggccaagagcatccctctgcgcagacaggtgtctgctgactccagtgcatccatgaactctggggttcttctggttcggccatcacggctctcctccagtgggactcccatgctagcaggggtctctgagtatgagcttcccgaagaccctcgctgggagctgcctcgggacagactggtcttaggcaaacccctgggagagggctgctttgggcaggtggtgttggcagaggctatcgggctggacaaggacaaacccaaccgtgtgaccaaagtggctgtgaagatgttgaagtcggacgcaacagagaaagacttgtcagacctgatctcagaaatggagatgatgaagatgatcgggaagcataagaatatcatcaacctgctgggggcctgcacgcaggatggtcccttgtatgtcatcgtggagtatgcctccaagggcaacctgcgggagtacctgcaggcccggaggcccccagggctggaatactgctacaaccccagccacaacccagaggagcagctctcctccaaggacctggtgtcctgcgcctaccaggtggcccgaggcatggagtatctggcctccaagaagtgcatacaccgagacctggcagccaggaatgtcctggtgacagaggacaatgtgatgaagatagcagactttggcctcgcacgggacattcaccacatcgactactataaaaagacaaccaacggccgactgcctgtgaagtggatggcacccgaggcattatttgaccggatctacacccaccagagtgatgtgtggtctttcggggtgctcctgtgggagatcttcactctgggcggctccccataccccggtgtgcctgtggaggaacttttcaagctgctgaaggagggtcaccgcatggacaagcccagtaactgcaccaacgagctgtacatgatgatgcgggactgctggcatgcagtgccctcacagagacccaccttcaagcagctggtggaagacctggaccgcatcgtggccttgacctccaaccaggagtacctggacctgtccatgcccctggaccagtactcccccagctttcccgacacccggagctctacgtgctcctcaggggaggattccgtcttctctcatgagccgctgcccgaggagccctgcctgccccgacacccagcccagcttgccaatggcggactcaaacgccgctga

SEQ ID NO: 17 - DNA, 20 bp, Homo sapiens
ttggacatccccagaaaaga

SEQ ID NO: 18 - DNA, 20 bp, Homo sapiens
ccatattggacatccccaga

SEQ ID NO: 19 - protein, 660 aa, Homo sapiens
MEKKLHAVPAAKTVKFKCPSSGTPNPTLRWLKNGKEFKPDHRIGGYKVRYATWSIIMDSVVPSDKGNYTCIVENEYGSINHTYQLDVVERSPHRPILQAGLPANKTVALGSNVEFMCKVYSDPQPHIQWLKHIEVNGSKIGPDNLPYVQILKTAGVNTTDKEMEVLHLRNVSFEDAGEYTCLAGNSIGLSHHSAWLTVLEALEERPAVMTSPLYLEIIIYCTGAFLISCMVGSVIVYKMKSGTKKSDFHSQMAVHKLAKSIPLRRQVSADSSASMNSGVLLVRPSRLSSSGTPMLAGVSEYELPEDPRWELPRDRLVLGKPLGEGCFGQVVLAEAIGLDKDKPNRVTKVAVKMLKSDATEKDLSDLISEMEMMKMIGKHKNIINLLGACTQDGPLYVIVEYASKGNLREYLQARRPPGLEYCYNPSHNPEEQLSSKDLVSCAYQVARGMEYLASKKCIHRDLAARNVLVTEDNVMKIADFGLARDIHHIDYYKKTTNGRLPVKWMAPEALFDRIYTHQSDVWSFGVLLWEIFTLGGSPYPGVPVEELFKLLKEGHRMDKPSNCTNELYMMMRDCWHAVPSQRPTFKQLVEDLDRIVALTSNQEYLDLSMPLDQYSPSFPDTRSSTCSSGEDSVFSHEPLPEEPCLPRHPAQLANGGLKRR

SEQ ID NO: 20 - DNA, 2431 bp, Homo sapiens
actgctggagttaataccaccgacaaagagatggaggtgcttcacttaagaaatgtctcctttgaggacgcaggggagtatacgtgcttggcgggtaactctatcggactctcccatcactctgcatggttgaccgttctggaagccctggaagagaggccggcagtgatgacctcgcccctgtacctggagatcatcatctattgcacaggggccttcctcatctcctgcatggtggggtcggtcatcgtctacaagatgaagagtggtaccaagaagagtgacttccacagccagatggctgtgcacaagctggccaagagcatccctctgcgcagacaggtaacagtgtctgctgactccagtgcatccatgaactctggggttcttctggttcggccatcacggctctcctccagtgggactcccatgctagcaggggtctctgagtatgagcttcccgaagaccctcgctgggagctgcctcgggacagactggtcttaggcaaacccctgggagagggctgctttgggcaggtggtgttggcagaggctatcgggctggacaaggacaaacccaaccgtgtgaccaaagtggctgtgaagatgttgaagtcggacgcaacagagaaagacttgtcagacctgatctcagaaatggagatgatgaagatgatcgggaagcataagaatatcatcaacctgctgggggcctgcacgcaggatggtcccttgtatgtcatcgtggagtatgcctccaagggcaacctgcgggagtacctgcaggcccggaggcccccagggctggaatactgctacaaccccagccacaacccagaggagcagctctcctccaaggacctggtgtcctgcgcctaccaggtggcccgaggcatggagtatctggcctccaagaagtgcatacaccgagacctggcagccaggaatgtcctggtgacagaggacaatgtgatgaagatagcagactttggcctcgcacgggacattcaccacatcgactactataaaaagacaaccaacggccgactgcctgtgaagtggatggcacccgaggcattatttgaccggatctacacccaccagagtgatgtgtggtctttcggggtgctcctgtgggagatcttcactctgggcggctccccataccccggtgtgcctgtggaggaacttttcaagctgctgaaggagggtcaccgcatggacaagcccagtaactgcaccaacgagctgtacatgatgatgcgggactgctggcatgcagtgccctcacagagacccaccttcaagcagctggtggaagacctggaccgcatcgtggccttgacctccaaccaggagtacctggacctgtccatgcccctggaccagtactcccccagctttcccgacacccggagctctacgtgctcctcaggggaggattccgtcttctctcatgagccgctgcccgaggagccctgcctgccccgacacccagcccagcttgccaatggcggactcaaacgccgctgactgccacccacacgccctccccagactccaccgtcagctgtaaccctcacccacagcccctgctgggcccaccacctgtccgtccctgtcccctttcctgctggcaggagccggctgcctaccaggggccttcctgtgtggcctgccttcaccccactcagctcacctctccctccacctcctctccacctgctggtgagaggtgcaaagaggcagatctttgctgccagccacttcatcccctcccagatgttggaccaacacccctccctgccaccaggcactgcctggagggcagggagtgggagccaatgaacaggcatgcaagtgagagcttcctgagctttctcctgtcggtttggtctgttttgccttcacccataagcccctcgcactctggtggcaggtgccttgtcctcagggctacagcagtagggaggtcagtgcttcgtgcctcgattgaaggtgacctctgccccagataggtggtgccagtggcttattaattccgatactagtttgctttgctgaccaaatgcctggtaccagaggatggtgaggcgaaggccaggttgggggcagtgttgtggccctggggcccagccccaaactgggggctctgtatatagctatgaagaaaacacaaagtgtataaatctgagtatatatttacatgtctttttaaaagggtcgttaccagagatttacccatcgggtaagatgctcctggtggctgggaggcatcagttgctatatattaaaaacaaaaaagaaaaaaaaggaaaatgtttttaaaaaggtcatatattttttgctacttttgctgttttatttttttaaattatgttctaaacctattttcagtttaggtccctcaataaaaattgctgctgcttca

SEQ ID NO: 21 - DNA, 1503 bp, Homo sapiens
atggaggtgcttcacttaagaaatgtctcctttgaggacgcaggggagtatacgtgcttggcgggtaactctatcggactctcccatcactctgcatggttgaccgttctggaagccctggaagagaggccggcagtgatgacctcgcccctgtacctggagatcatcatctattgcacaggggccttcctcatctcctgcatggtggggtcggtcatcgtctacaagatgaagagtggtaccaagaagagtgacttccacagccagatggctgtgcacaagctggccaagagcatccctctgcgcagacaggtaacagtgtctgctgactccagtgcatccatgaactctggggttcttctggttcggccatcacggctctcctccagtgggactcccatgctagcaggggtctctgagtatgagcttcccgaagaccctcgctgggagctgcctcgggacagactggtcttaggcaaacccctgggagagggctgctttgggcaggtggtgttggcagaggctatcgggctggacaaggacaaacccaaccgtgtgaccaaagtggctgtgaagatgttgaagtcggacgcaacagagaaagacttgtcagacctgatctcagaaatggagatgatgaagatgatcgggaagcataagaatatcatcaacctgctgggggcctgcacgcaggatggtcccttgtatgtcatcgtggagtatgcctccaagggcaacctgcgggagtacctgcaggcccggaggcccccagggctggaatactgctacaaccccagccacaacccagaggagcagctctcctccaaggacctggtgtcctgcgcctaccaggtggcccgaggcatggagtatctggcctccaagaagtgcatacaccgagacctggcagccaggaatgtcctggtgacagaggacaatgtgatgaagatagcagactttggcctcgcacgggacattcaccacatcgactactataaaaagacaaccaacggccgactgcctgtgaagtggatggcacccgaggcattatttgaccggatctacacccaccagagtgatgtgtggtctttcggggtgctcctgtgggagatcttcactctgggcggctccccataccccggtgtgcctgtggaggaacttttcaagctgctgaaggagggtcaccgcatggacaagcccagtaactgcaccaacgagctgtacatgatgatgcgggactgctggcatgcagtgccctcacagagacccaccttcaagcagctggtggaagacctggaccgcatcgtggccttgacctccaaccaggagtacctggacctgtccatgcccctggaccagtactcccccagctttcccgacacccggagctctacgtgctcctcaggggaggattccgtcttctctcatgagccgctgcccgaggagccctgcctgccccgacacccagcccagcttgccaatggcggactcaaacgccgctga

SEQ ID NO: 22 - DNA, 20 bp, Homo sapiens
ccgacaaagagatggaggtg

SEQ ID NO: 23 - DNA, 22 bp, Homo sapiens
caaagagatggaggtgcttcac

SEQ ID NO: 24 - protein, 452 aa, Homo sapiens [sequence omitted]

SEQ ID NO: 25 - DNA, 1296 bp, Homo sapiens
atggtggggtcggtcatcgtctacaagatgaagagtggtaccaagaagagtgacttccacagccagatggctgtgcacaagctggccaagagcatccctctgcgcagacaggtgtctgctgactccagtgcatccatgaactctggggttcttctggttcggccatcacggctctcctccagtgggactcccatgctagcaggggtctctgagtatgagcttcccgaagaccctcgctgggagctgcctcgggacagactggtcttaggcaaacccctgggagagggctgctttgggcaggtggtgttggcagaggctatcgggctggacaaggacaaacccaaccgtgtgaccaaagtggctgtgaagatgttgaagtcggacgcaacagagaaagacttgtcagacctgatctcagaaatggagatgatgaagatgatcgggaagcataagaatatcatcaacctgctgggggcctgcacgcaggatggtcccttgtatgtcatcgtggagtatgcctccaagggcaacctgcgggagtacctgcaggcccggaggcccccagggctggaatactgctacaaccccagccacaacccagaggagcagctctcctccaaggacctggtgtcctgcgcctaccaggtggcccgaggcatggagtatctggcctccaagaagtgcatacaccgagacctggcagccaggaatgtcctggtgacagaggacaatgtgatgaagatagcagactttggcctcgcacgggacattcaccacatcgactactataaaaagacaaccaacggccgactgcctgtgaagtggatggcacccgaggcattatttgaccggatctacacccaccagagtgatgtgtggtctttcggggtgctcctgtgggagatcttcactctgggcggctccccataccccggtgtgcctgtggaggaacttttcaagctgctgaaggagggtcaccgcatggacaagcccagtaactgcaccaacgagctgtacatgatgatgcgggactgctggcatgcagtgccctcacagagacccaccttcaagcagctggtggaagacctggaccgcatcgtggccttgacctccaaccaggagtacctggacctgtccatgcccctggaccagtactcccccagctttcccgacacccggagctctacgtgctcctcaggggaggattccgtcttctctcatgagccgctgcccgaggagccctgcctgccccgacacccagcccagcttgccaatggcggactcaaacgccgctga

SEQ ID NO: 26 - protein, 431 aa, Homo sapiens [sequence omitted]

SEQ ID NO: 27 - DNA, 17 bp, Homo sapiens
atggtggggtcggtcat

SEQ ID NO: 28 - DNA, 1269 bp, Homo sapiens
atgaagagtggtaccaagaagagtgacttccacagccagatggctgtgcacaagctggccaagagcatccctctgcgcagacaggtgtctgctgactccagtgcatccatgaactctggggttcttctggttcggccatcacggctctcctccagtgggactcccatgctagcaggggtctctgagtatgagcttcccgaagaccctcgctgggagctgcctcgggacagactggtcttaggcaaacccctgggagagggctgctttgggcaggtggtgttggcagaggctatcgggctggacaaggacaaacccaaccgtgtgaccaaagtggctgtgaagatgttgaagtcggacgcaacagagaaagacttgtcagacctgatctcagaaatggagatgatgaagatgatcgggaagcataagaatatcatcaacctgctgggggcctgcacgcaggatggtcccttgtatgtcatcgtggagtatgcctccaagggcaacctgcgggagtacctgcaggcccggaggcccccagggctggaatactgctacaaccccagccacaacccagaggagcagctctcctccaaggacctggtgtcctgcgcctaccaggtggcccgaggcatggagtatctggcctccaagaagtgcatacaccgagacctggcagccaggaatgtcctggtgacagaggacaatgtgatgaagatagcagactttggcctcgcacgggacattcaccacatcgactactataaaaagacaaccaacggccgactgcctgtgaagtggatggcacccgaggcattatttgaccggatctacacccaccagagtgatgtgtggtctttcggggtgctcctgtgggagatcttcactctgggcggctccccataccccggtgtgcctgtggaggaacttttcaagctgctgaaggagggtcaccgcatggacaagcccagtaactgcaccaacgagctgtacatgatgatgcgggactgctggcatgcagtgccctcacagagacccaccttcaagcagctggtggaagacctggaccgcatcgtggccttgacctccaaccaggagtacctggacctgtccatgcccctggaccagtactcccccagctttcccgacacccggagctctacgtgctcctcaggggaggattccgtcttctctcatgagccgctgcccgaggagccctgcctgccccgacacccagcccagcttgccaatggcggactcaaacgccgctga

SEQ ID NO: 29 - protein, 422 aa, Homo sapiens
MKSGTKKSDFHSQMAVHKLAKSIPLRRQVSADSSASMNSGVLLVRPSRLSSSGTPMLAGVSEYELPEDPRWELPRDRLVLGKPLGEGCFGQVVLAEAIGLDKDKPNRVTKVAVKMLKSDATEKDLSDLISEMEMMKMIGKHKNIINLLGACTQDGPLYVIVEYASKGNLREYLQARRPPGLEYCYNPSHNPEEQLSSKDLVSCAYQVARGMEYLASKKCIHRDLAARNVLVTEDNVMKIADFGLARDIHHIDYYKKTTNGRLPVKWMAPEALFDRIYTHQSDVWSFGVLLWEIFTLGGSPYPGVPVEELFKLLKEGHRMDKPSNCTNELYMMMRDCWHAVPSQRPTFKQLVEDLDRIVALTSNQEYLDLSMPLDQYSPSFPDTRSSTCSSGEDSVFSHEPLPEEPCLPRHPAQLANGGLKRR

SEQ ID NO: 30 - DNA, 25 bp, Homo sapiens
atgaagagtggtaccaagaagagtg

SEQ ID NO: 31 - DNA, 1104 bp, Homo sapiens
atgctagcaggggtctctgagtatgagcttcccgaagaccctcgctgggagctgcctcgggacagactggtcttaggcaaacccctgggagagggctgctttgggcaggtggtgttggcagaggctatcgggctggacaaggacaaacccaaccgtgtgaccaaagtggctgtgaagatgttgaagtcggacgcaacagagaaagacttgtcagacctgatctcagaaatggagatgatgaagatgatcgggaagcataagaatatcatcaacctgctgggggcctgcacgcaggatggtcccttgtatgtcatcgtggagtatgcctccaagggcaacctgcgggagtacctgcaggcccggaggcccccagggctggaatactgctacaaccccagccacaacccagaggagcagctctcctccaaggacctggtgtcctgcgcctaccaggtggcccgaggcatggagtatctggcctccaagaagtgcatacaccgagacctggcagccaggaatgtcctggtgacagaggacaatgtgatgaagatagcagactttggcctcgcacgggacattcaccacatcgactactataaaaagacaaccaacggccgactgcctgtgaagtggatggcacccgaggcattatttgaccggatctacacccaccagagtgatgtgtggtctttcggggtgctcctgtgggagatcttcactctgggcggctccccataccccggtgtgcctgtggaggaacttttcaagctgctgaaggagggtcaccgcatggacaagcccagtaactgcaccaacgagctgtacatgatgatgcgggactgctggcatgcagtgccctcacagagacccaccttcaagcagctggtggaagacctggaccgcatcgtggccttgacctccaaccaggagtacctggacctgtccatgcccctggaccagtactcccccagctttcccgacacccggagctctacgtgctcctcaggggaggattccgtcttctctcatgagccgctgcccgaggagccctgcctgccccgacacccagcccagcttgccaatggcggactcaaacgccgctga

SEQ ID NO: 32 - protein, 367 aa, Homo sapiens
MLAGVSEYELPEDPRWELPRDRLVLGKPLGEGCFGQVVLAEAIGLDKDKPNRVTKVAVKMLKSDATEKDLSDLISEMEMMKMIGKHKNIINLLGACTQDGPLYVIVEYASKGNLREYLQARRPPGLEYCYNPSHNPEEQLSSKDLVSCAYQVARGMEYLASKKCIHRDLAARNVLVTEDNVMKIADFGLARDIHHIDYYKKTTNGRLPVKWMAPEALFDRIYTHQSDVWSFGVLLWEIFTLGGSPYPGVPVEELFKLLKEGHRMDKPSNCTNELYMMMRDCWHAVPSQRPTFKQLVEDLDRIVALTSNQEYLDLSMPLDQYSPSFPDTRSSTCSSGEDSVFSHEPLPEEPCLPRHPAQLANGGLKRR

SEQ ID NO: 33 - DNA, 19 bp, Homo sapiens
catgctagcaggggtctct

SEQ ID NO: 34 - DNA, 1104 bp, Homo sapiens; identical to SEQ ID NO: 31

SEQ ID NO: 35 - protein, 308 aa, Homo sapiens
MLKSDATEKDLSDLISEMEMMKMIGKHKNIINLLGACTQDGPLYVIVEYASKGNLREYLQARRPPGLEYCYNPSHNPEEQLSSKDLVSCAYQVARGMEYLASKKCIHRDLAARNVLVTEDNVMKIADFGLARDIHHIDYYKKTTNGRLPVKWMAPEALFDRIYTHQSDVWSFGVLLWEIFTLGGSPYPGVPVEELFKLLKEGHRMDKPSNCTNELYMMMRDCWHAVPSQRPTFKQLVEDLDRIVALTSNQEYLDLSMPLDQYSPSFPDTRSSTCSSGEDSVFSHEPLPEEPCLPRHPAQLANGGLKRR

SEQ ID NO: 36 - DNA, 20 bp, Homo sapiens
atgctagcaggggtctctga

SEQ ID NO: 37 - DNA, 2463 bp, Homo sapiens
atgtggagctggaagtgcctcctcttctgggctgtgctggtcacagccacactctgcaccgctaggccgtccccgaccttgcctgaacaagcccagccctggggagcccctgtggaagtggagtccttcctggtccaccccggtgacctgctgcagcttcgctgtcggctgcgggacgatgtgcagagcatcaactggctgcgggacggggtgcagctggcggaaagcaaccgcacccgcatcacaggggaggaggtggaggtgcaggactccgtgcccgcagactccggcctctatgcttgcgtaaccagcagcccctcgggcagtgacaccacctacttctccgtcaatgtttcagatgctctcccctcctcggaggatgatgatgatgatgatgactcctcttcagaggagaaagaaacagataacaccaaaccaaaccccgtagctccatattggacatccccagaaaagatggaaaagaaattgcatgcagtgccggctgccaagacagtgaagttcaaatgcccttccagtgggaccccaaaccccacactgcgctggttgaaaaatggcaaagaattcaaacctgaccacagaattggaggctacaaggtccgttatgccacctggagcatcataatggactctgtggtgccctctgacaagggcaactacacctgcattgtggagaatgagtacggcagcatcaaccacacataccagctggatgtcgtggagcggtcccctcaccggcccatcctgcaagcagggttgcccgccaacaaaacagtggccctgggtagcaacgtggagttcatgtgtaaggtgtacagtgacccgcagccgcacatccagtggctaaagcacatcgaggtgaatgggagcaagattggcccagacaacctgccttatgtccagatcttgaagactgctggagttaataccaccgacaaagagatggaggtgcttcacttaagaaatgtctcctttgaggacgcaggggagtatacgtgcttggcgggtaactctatcggactctcccatcactctgcatggttgaccgttctggaagccctggaagagaggccggcagtgatgacctcgcccctgtacctggagatcatcatctattgcacaggggccttcctcatctcctgcatggtggggtcggtcatcgtctacaagatgaagagtggtaccaagaagagtgacttccacagccagatggctgtgcacaagctggccaagagcatccctctgcgcagacaggtaacagtgtctgctgactccagtgcatccatgaactctggggttcttctggttcggccatcacggctctcctccagtgggactcccatgctagcaggggtctctgagtatgagcttcccgaagaccctcgctgggagctgcctcgggacagactggtcttaggcaaacccctgggagagggctgctttgggcaggtggtgttggcagaggctatcgggctggacaaggacaaacccaaccgtgtgaccaaagtggctgtgaagatgttgaagtcggacgcaacagagaaagacttgtcagacctgatctcagaaatggagatgatgaagatgatcgggaagcataagaatatcatcaacctgctgggggcctgcacgcaggatggtcccttgtatgtcatcgtggagtatgcctccaagggcaacctgcgggagtacctgcaggcccggaggcccccagggctggaatactgctacaaccccagccacaacccagaggagcagctctcctccaaggacctggtgtcctgcgcctaccaggtggcccgaggcatggagtatctggcctccaagaagtgcatacaccgagacctggcagccaggaatgtcctggtgacagaggacaatgtgatgaagatagcagactttggcctcgcacgggacattcaccacatcgactactataaaaagacaaccaacggccgactgcctgtgaagtggatggcacccgaggcattatttgaccggatctacacccaccagagtgatgtgtggtctttcggggtgctcctgtgggagatcttcactctgggcggctccccataccccggtgtgcctgtggaggaacttttcaagctgctgaaggagggtcaccgcatggacaagcccagtaactgcaccaacgagctgtacatgatgatgcgggactgctggcatgcagtgccctcacagagacccaccttcaagcagctggtggaagacctggaccgcatcgtggccttgacctccaaccaggagtacctggacctgtccatgcccctggaccagtactcccccagctttcccgacacccggagctctacgtgctcctcaggggaggattccgtcttctctcatgagccgctgcccgaggagccctgcctgccccgacacccagcccagcttgccaatggcggactcaaacgccgctga